European Patent Application EP 4 198 135 A1, published June 21, 2023. Title: Nucleic acid construct for increasing adeno-associated virus yield, and construction method therefor. Applicant: Hangzhou Geneway Biotechnology Co., Ltd. The sequence listing filed with the application follows.

SEQUENCE LISTING (22 sequences)

SEQ ID NO: 1 - DNA, 14057 bp, Artificial sequence
  Nucleotide sequence of nucleic acid construct
ttctctgtcacagaatgaaaatttttctgtcatctcttcgttattaatgtttgtaattgactgaatatcaacgcttatttgcagcctgaatggcgaatgggacgcgccctgtagcggcgcattaagcgcggcgggtgtggtggttacgcgcagcgtgaccgctacacttgccagcgccctagcgcccgctcctttcgctttcttcccttcctttctcgccacgttcgccggctttccccgtcaagctctaaatcgggggctccctttagggttccgatttagtgctttacggcacctcgaccccaaaaaacttgattagggtgatggttcacgtagtgggccatcgccctgatagacggtttttcgccctttgacgttggagtccacgttctttaatagtggactcttgttccaaactggaacaacactcaaccctatctcggtctattcttttgatttataagggattttgccgatttcggcctattggttaaaaaatgagctgatttaacaaaaatttaacgcgaattttaacaaaatattaacgtttacaatttcaggtggcacttttcggggaaatgtgcgcggaacccctatttgtttatttttctaaatacattcaaatatgtatccgctcatgagacaataaccctgataaatgcttcaataatattgaaaaaggaagagtatgagtattcaacatttccgtgtcgcccttattcccttttttgcggcattttgccttcctgtttttgctcacccagaaacgctggtgaaagtaaaagatgctgaagatcagttgggtgcacgagtgggttacatcgaactggatctcaacagcggtaagatccttgagagttttcgccccgaagaacgttttccaatgatgagcacttttaaagttctgctatgtggcgcggtattatcccgtattgacgccgggcaagagcaactcggtcgccgcatacactattctcagaatgacttggttgagtactcaccagtcacagaaaagcatcttacggatggcatgacagtaagagaattatgcagtgctgccataaccatgagtgataacactgcggccaacttacttctgacaacgatcggaggaccgaaggagctaaccgcttttttgcacaacatgggggatcatgtaactcgccttgatcgttgggaaccggagctgaatgaagccataccaaacgacgagcgtgacaccacgatgcctgtagcaatggcaacaacgttgcgcaaactattaactggcgaactacttactctagcttcccggcaacaattaatagactggatggaggcggataaagttgcaggaccacttctgcgctcggcccttccggctggctggtttattgctgataaatctggagccggtgagcgtgggtctcgcggtatcattgcagcactggggccagatggtaagccctcccgtatcgtagttatctacacgacggggagtcaggcaactatggatgaacgaaatagacagatcgctgagataggtgcctcactgattaagcattggtaactgtcagaccaagtttactcatatatactttagattgatttaaaacttcatttttaatttaaaaggatctaggtgaagatcctttttgataatctcatgaccaaaatcccttaacgtgagttttcgttccactgagcgtcagaccccgtagaaaagatcaaaggatcttcttgagatcctttttttctgcgcgtaatctgctgcttgcaaacaaaaaaaccaccgctaccagcggtggtttgtttgccggatcaagagctaccaactctttttccgaaggtaactggcttcagcagagcgcagataccaaatactgtccttctagtgtagccgtagttaggccaccacttcaagaactctgtagcaccgcctacatacctcgctctgctaatcctgttaccagtggctgctgccagtggcgataagtcgtgtcttaccgggttggactcaagacgatagttaccggataaggcgcagcggtcgggctgaacggggggttcgtgcacacagcccagcttggagcgaacgacctacaccgaactgagatacctacagcgtgagcattgagaaagcgccacgcttcccgaagggagaaaggcggacaggtatccggtaagcggcagggtcggaacaggagagcgcacgagggagcttccagggggaaacgcctggtatctttatagtcctgtcgggtttcgccacctctgacttgagcgtcgatttttgtgatgctcgtcaggggggcggagcctatggaaaaacgccagcaacgcggcctttttacggttcctggccttttgctggccttttgctcacatgttctttcctgcgttatcccctgattctgtggataaccgtattaccgcctttgagtgagctgataccgctcgccgcagccgaacgaccgagcgcagcgagtcagtgagcgaggaagcggaagagcgcctgatgcggtattttctccttacgcatctgtgcggtatttcacaccgcagaccagccgcgtaacctggcaaaatcggttacggttgagtaataaatggatgccctgcgtaagcgggtgtgggcggacaataaagtcttaaactgaacaaaatagatctaaactatgacaataaagtcttaaactagacagaatagttgtaaactgaaatcagtccagttatgctgtgaaaaagcatactggacttttgttatggctaaagcaaactcttcattttctgaagtgcaaattgcccgtcgtattaaagaggggcgtggccaagggcatggtaaagactatattcgcggcgttgtgacaatttaccgaacaactccgcggccgggaagccgatctcggcttgaacgaattgttaggtggcggtacttgggtcgatatcaaagtgcatcacttcttcccgtatgcccaactttgtatagagagccactgcgggatcgtcaccgtaatctgcttgcacgtagatcacataagcaccaagcgcgttggcctcatgcttgaggagattgatgagcgcggtggcaatgccctgcctccggtgctcgccggagactgcgagatcatagatatagatctcactacgcggctgctcaaacctgggcagaacgtaagccgcgagagcgccaacaaccgcttcttggtcgaaggcagcaagcgcgatgaatgtcttactacggagcaagttcccgaggtaatcggagtccggctgatgttgggagtaggtggctacgtctccgaactcacgaccgaaaagatcaagagcagcccgcatggatttgacttggtcagggccgagcctacatgtgcgaatgatgcccatacttgagccacctaactttgttttagggcgactgccctgctgcgtaacatcgttgctgctgcgtaacatcgttgctgctccataacatcaaacatcgacccacggcgtaacgcgcttgctgcttggatgcccgaggcatagactgtacaaaaaaacagtcataacaagccatgaaaaccgccactgcgccgttaccaccgctgcgttcggtcaaggttctggaccagttgcgtgagcgcatacgctacttgcattacagtttacgaaccgaacaggcttatgtcaactgggttcgtgccttcatccgtttccacggtgtgcgtcacccggcaaccttgggcagcagcgaagtcgaggcatttctgtcctggctggcgaacgagcgcaaggtttcggtctccacgcatcgtcaggcattggcggccttgctgttcttctacggcaaggtgctgtgcacggatctgccctggcttcaggagatcggtagacctcggccgtcgcggcgcttgccggtggtgctgaccccggatgaagtggttcgcatcctcggttttctggaaggcgagcatcgtttgttcgcccaggactctagctatagttctagtggttggcctacgtacccgtagtggctatggcagggcttgccgccccgacgttggctgcgagccctgggccttcacccgaacttgggggttggggtggggaaaaggaagaaacgcgggcgtattggtcccaatggggtctcggtggggtatcgacagagtgccagccctgggaccgaaccccgcgtttatgaacaaacgacccaacacccgtgcgttttattctgtctttttattgccgtcatagcgcgggttccttccggtattgtctccttccgtgtttcagttagcctcccccatctcccggtaccgcatgccttagttgaactcgaacttcttgtacttgcagttgagcttttgctcggcgaatgtgatggcgtcggagagtggcaccagtccctgcaggatcaaggccaagagcttcagcaagttgttgtgcagtgtagttgactcgcgacggttgaccttgccgatcacgaacatgtggtgcttgaatctgttgtacttttggatgacctggctcacatcaacgtccttgatttcgccagagatccagtagaactccttgttcttcttagcgatggtcagcctttcctcgttcttgaaggacaacacgatgaagttgtgacccttaacgttatcgacgttttgagtcaagtactgctcaacgatgtgcatgcttccgtcttccttcttgaccttcttgaggttctcggcgttgttgttagaagcgatgttgtcgtggtacttgtagttgttgaagagcaggttagcgacggacgagtacttgtatgtcagagtgctcttcttgttcacgatgaggttcaggttatcaacgacgtacttgttgggagggttgtccgggaattggacggactccgagtacttgaggatctgggaaacgtatggcgagacgaagaagttgttagaggcggtttcgatctcgtttgattccttgcggctcagcatgatgggcaaagtgaagaggttcttgtcctggtacatctcgtacaacttcgacaagaggaatccacacttacgctcgccgagtgattgcagcaaggtcacgaaggttgtctgagcgtagtacatatcgaggttgaagtaggaggtcagagcggccttgaatgtgtggtggacgtccacgaagtgacacttcttgcagttttgagcggcggtctcatcgttgcagacgtcctgtgagtgtgggatttcgatgccagtctccttaaccaggttgtagctgatcatgaagcggatcttatcgaaggtcacaacgaacacacggttgtcaaccatgtagtagttgtttgtgtactcgtagaccacgttagagacgtacttggcgaagatgatttcgaaaggcttcacctcggacttcttaacgacgaacatgtagtaaccggtttcagacatgtgatcggagaatctgttcgagttgtagtcgttatcgtcgaacctcatcaggtagggggcgaagtcgtttgtgaagtagtgagtgatctcctgggtggaagccactgtacagatgttagtgttgtggttgatggtttgttccagtgtagcgcatgactggatggtgctcttcttgtacttaggtctcaacttgatcttgttgaattgacccacaactccctgggagttatccaggtactcgtccaacttcctcttggtgcctgtggccgacggctggttgacaccagcagagtgttcgaaggactcggcgtggtaagctgagctaggagagggttgttcgaccactggctgttcgagtgactcgctgtagtaggcagaggacacagcttcctccaggttgtcagtggtcttgagcagacactccaccaaatcgttgtcagtgagcgagttaactgaggcgaggaagttgctagcggcagcggtttcagagtcggagatgacagtatcagctccgtccggggttgggtggttgtagtaagacaagtaatcgttaggttgcttgtcgcagaactccgagtatgagttgtcgaagctagcacgagagggagtgctggcagaggtgtaggaagcgttgaagttgatttgagtcatggtgacctggttgttcacgatcttatcgccacctgtgtccacctgcagttgctgggcctcagcgcaggctgaagtggcctcacaggagtaggggctggaagcacagttggaagtcatgatgttttcttggacgttcaggacgtggctggatgtacggatcatgcgcccgatggtgggacggtatgaataatccggaatatttataggtttttttattacaaaactgttacgaaaacagtaaaatacttatttatttgcgagatggttatcattttaattatctccatgatcggatctcctaggctcaagcagtgatcagatccagacatgataagatacattgatgagtttggacaaaccacaactagaatgcagtgaaaaaaatgctttatttgtgaaatttgtgatgctattgctttatttgtaaccattataagctgcaataaacaagttaacaacaacaattgcatttgtctagtacttctcgacggtaccgcatgctatgcatcagctgctagcaccatggctcgagttacagattacgagtcaggtatctggtgccaatggggcgaggctctgaatacacgccattagtgtccacagtaaagtccacattaacagacttgttgtagttggaagtgtactgaatttcgggattccagcgtttgctgttttccttctgcagctcccactcgatctccacgctgacctgtcccgtggagtactgtgtgatgaaggaagcaaactttgccgcactgaaggtggtcgaaggattcgcaggtaccggggtgttcttgatgagaatctgtggaggagggtgtttaagtccgaatccacccatgaggggagaggggtgaaaatgtccgtccgtgtgtggaatctttgcccagatgggcccctgaaggtacacatctctgtcctgccagaccatgcctggaagaacgccttgtgtgttgacatctgcggtagctgcttgtctgttgcctctctggaggttggtagatacagaaccatactgctccgtagccacgggattggttgtcctgatttcctcttcgtctgtaatcatgaccttttcaatgtccacatttgttttctctgagccttgcttcccaaagatgagaaccccgctctgaggaaaaaacttttcttcatcgtccttgtggcttgccatcgccgggcccggattcaccagagagtctctgccattgaggtggtacttggtagctccagtccacgagtattcactgttgttgttatccgcagatgtctttgatactcgctgctggcggtaacagggtccaggaagccagttcctagactggtcccgaatgtcactcgctccggcctgagaaaactgaagccttgactgcgtggtggttccacttggagtgtttgttctgctcaagtaatacaggtactggtcgatgagaggattcatgagacggtccagactctggctgtgagcgtagctgctgtggaaaggaacgtcctcaaaagtgtagctgaaggtaaagttgtttccggtacgcagcatctgagaaggaaagtactccaggcagtaaaatgaagagcgtcctactgcctgactcccgttgttcagggtgaggtatccatactgtggcaccatgaagacgtctgctgggaacggcgggaggcatccttgatgcgccgagccgaggacgtacgggagctggtactccgagtcagtaaacacctgaaccgtgctggtaaggttattggcaatcgtcgtcgtaccgtcattctgcgtgacctctttgacttgaatgttaaagagcttgaagttgagtctcttgggtcggaatccccagttgttgttgatgagtctttgccagtcacgtggtgaaaagtggcagtggaatctgttgaagtcaaaatacccccaaggggtgctgtagccaaagtagtgattgtcgttcgaggctcctgattggctggaaatttgtttgtagaggtggttgttgtaggtgggcagggcccaggttcgggtgctggtggtgatgactctgtcgcccatccatgtggaatcgcaatgccaatttcccgaggaattacccactccgtcggcgccctcgttattgtctgccattggtgcgccactgcctgtagccatcgtattagttcccagaccagagggggctgctggtggctgtccgagaggctgggggtcaggtactgagtctgcgtctccagtctgaccaaaattcaatctttttcttgcaggctgctggcccgcctttccggttcccgaggaggagtctggctccacaggagagtgctctaccggcctcttttttcccggagccgtcttaacaggttcctcaaccaggcccagaggttcaagaaccctctttttcgcctggaagactgctcgtccgaggttgcccccaaaagacgtatcttctttaaggcgctcctggaactccgcgtcggcgtggttgtacttgaggtaagggttgtctccgctgtcgagctgccggtcgtaggctttgtcgtgctcgagggcagcggcgtctgcctcgttcaccggctctcccttgtccagtccgttgaagggtccgaggtacttgtacccgggaagcacaaggcccctgctgtcgtccttatgccgctctgcgggctttggtggtggtgggccgggtttgagcttccaccactgtcttattccttcagagagagtgtcctcgagccaatcgggtagataaccgtcggcagccgtggcggctcaagtcttcgtcgagtgattgtaaataaaatgtaatttacagtatagtattttaattaatatacaaatgatttgataataattcttatttaactataatatattgtgttgggttgaattaaaggtccgtatctccagactgcagtttaaattgtgtaatttatgtagctgtaatttttaccttattaatattttttacgctttgcattcgacgactgaactcccaaatatatgtttaactcgtcttggtcgtttgaatttttgttgctgtgtttcctaatattttccatcaccttaaatatgttattgtaatcctcaatgttgaacttgcaattggacacggcatagttttccatagtcgtgtaaaacatggtattggctgcattgtaatacatccgactgagcgggtacggatctatgtgtttgagcagcctgttcaaaaactctgcatcgtcgcaaaacggaatttggtcacgatcccggtccgaagcgcgcggaattcaaagcgctacgtcagcgacgtcatcgattattgctccaatactagggttttgttttactatctgttctgcggtccacacatcttcttcgctagtcacgtacgcaaacaactcgggccgcaaaggtgttttaaaacatatcagattagaatcttttataacttggccgcattgtaaatagttgtgccaacgcgcgggaaacattttacacgtgctttcaatcttatctcataaacgcaactaaatatgatccttcaactcgctttacgagtagaattctacttgtaacgcacgattaattatgactcataagctgatgtcatgttttgcacacggctcataaccgaactcgctttacgagtagaattctacgcgtaaaacacaatcaagtatgagtcataagctgatgtcatgttttgcacacggctcataaccgaactggctttacgagtagaattctacttgtaacgcacgatcagtggatgatgtcataaacttatctcatgttttgcacacggctcataacttgagtcataagctgatatcagaagattattaacgtgtttaggtatgactcatttgttttcaaaactgaactcgctttacggatagaattctacttgtaaaacacaatcaggggatgatgtcattatacaaatgatgtcatttgtttttcaaaactaaactcgctttacgggtagaattctacttgtaaaacacaatcgagggataatgtcatttgttattctcaaatatgatgtcatttaaatttttattatgcaagaattgtatgttgctgtgtcatttatgaatgttttatcgacaacttgtttatttgtttcattgacttgttgttgttcgtgattatgattaattataaatcttttgttggggtcaacatcgatgtatacgccgctacagggcgcgtactatggttgctttgacgtatgcggtgtgaaataccgcacagatgcgtaaggagaaaataccgcatcaggcgcccctgcaggcagctgcgcgctcgctcgctcactgaggccgcccgggcaaagcccgggcgtcgggcgacctttggtcgcccggcctcagtgagcgagcgagcgcgcagagagggagtggccaactccatcactaggggttcctacgcgttagttattaatagtaatcaattacggggtcattagttcatagcccatatatggagttccgcgttacataacttacggtaaatggcccgcctggctgaccgcccaacgacccccgcccattgacgtcaataatgacgtatgttcccatagtaacgccaatagggactttccattgacgtcaatgggtggagtatttacggtaaactgcccacttggcagtacatcaagtgtatcatatgccaagtacgccccctattgacgtcaatgacggtaaatggcccgcctggcattatgcccagtacatgaccttatgggactttcctacttggcagtacatctacgtattagtcatcgctattaccatggtgatgcggttttggcagtacatcaatgggcgtggatagcggtttgactcacggggatttccaagtctccaccccattgacgtcaatgggagtttgttttggcaccaaaatcaacgggactttccaaaatgtcgtaacaactccgccccattgacgcaaatgggcggtaggcgtgtacggtgggaggtctatataagcagagctggtttagtgaaccgtcagatccgctagcgctaccggtcgccaccgtcgacgtttatttgtgaaatttgtgatgctattgctttatttgtaaccatctagctttatttgtgaaatttgtgatgctattgctttatttgtaaccattataagctgcaataaacaagttaacaacaacaattgcattcattttatgtttcaggttcagggggagatgtgggaggttttttaaagtttaaacaggaacccctagtgatggagttggccactccctctctgcgcgctcgctcgctcactgaggccgggcgaccaaaggtcgcccgacgcccgggcggcctcagtgagcgagcgagcgcgcagctgcctgcaggacatgtgagcaaaaggccagcaaaaggccaggaaccgtaaaaaggccgcgttgctggcgtttttccataggctccgcccccctgacgagcatcacaaaaatcgacgctcgcggccgctctagagatcatggagataattaaaatgataaccatctcgcaaataaataagtattttactgttttcgtaacagttttgtaataaaaaaacctataaatattccggattattcataccgtcccaccatcgggcgcggatccgccgccctggcggggttttacgagattgtgattaaggtccccagcgaccttgacgagcatctgcccggcatttctgacagctttgtgaactgggtggccgagaaggagtgggagttgccgccagattctgacttggatctgaatctgattgagcaggcacccctgaccgtggccgagaagctgcagcgcgactttctgacggagtggcgccgtgtgagtaaggccccggaggcccttttctttgtgcaatttgagaagggagagagctacttccacttacacgtgctcgtggaaaccaccggggtgaaatccttagttttgggacgtttcctgagtcagattcgcgaaaaactgattcagagaatttaccgcgggatcgagccgactttgccaaactggttcgcggtcacaaagaccagaaacggcgccggaggcgggaacaaggtggtggacgagtgctacatccccaattacttgctccccaaaacccagcctgagctccagtgggcgtggactaatttagaacagtatttaagcgcctgtttgaatctcacggagcgtaaacggttggtggcgcagcatctgacgcacgtgtcgcagacgcaggagcagaacaaagagaatcagaatcccaattctgacgcgccggtgatcagatcaaaaacttcagccaggtacatggagctggtcgggtggctcgtggacaaggggattacctcggagaagcagtggatacaggaggaccaggcctcatacatctccttcaatgcggcctccaactcgcggtcccaaatcaaggctgccttggacaatgcgggaaagattatgagcctgactaaaaccgcccccgactacctggtgggccagcagcccgtggaggacatttccagcaatcggatttataaaattttggaactaaacgggtacgatccccaatatgcggcttccgtctttctgggatgggccacgaaaaagttcggcaagaggaacaccatctggctgtttgggcctgcaactaccgggaagaccaacatcgcggaggccatagcccacactgtgcccttctacgggtgcgtaaactggaccaatgagaactttcccttcaacgactgtgtggacaagatggtgatctggtgggaggaggggaagatgaccgccaaggtcgtggagtcggccaaagccattctcggaggaagcaaggtgcgcgtggaccagaaatgcaagtcctcggcccagatagacccgactcccgtgatcgtcacctccaacaccaacatgtgcgccgtgattgacgggaactcaacgaccttcgaacaccagcagccgttgcaagaccggatgttcaaatttgaactcacccgccgtctggatcatgactttgggaaggtcaccaagcaggaagtcaaagactttttccggtgggcaaaggatcacgtggttgaggtggagcatgaattctacgtcaaaaagggtggagccaagaaaagacccgcccccagtgacgcagatataagtgagcccaaacgggtgcgcgagtcagttgcgcagccatcgacgtcagacgcggaagcatcgatcaactacgcagacaggtaccaaaacaaatgttctcgtcacgtgggcatgaatctgatgctgtttccctgcagacaatgcgagagaatgaatcagaattcaaatatctgcttcactcacggacagaaagactgtttagagtgctttcccgtgtcagaatctcaacccgtttctgtcgtcaaaaaggcgtatcagaaactgtgctacattcatcatatcatgggaaaggtgccagacgcttgcactgcctgcgatctggtcaatgtggatttggatgactgcatctttgaacaataatctagagcctgcagtctcgacaagcttgtcgagaagtactagaggatcataatcagccataccacatttgtagaggttttacttgctttaaaaaacctcccacacctccccctgaacctgaaacataaaatgaatgcaattgttgttgttaacttgtttattgcagcttataatggttacaaataaagcaatagcatcacaaatttcacaaataaagcatttttttcactgcattctagttgtggtttgtccaaactcatcaatgtatcttatcatgtctggatctgatcactgcttgagcctaggagatccgaaccagataagtgaaatctagttccaaactattttgtcatttttaattttcgtattagcttacgacgctacacccagttcccatctattttgtcactcttccctaaataatccttaaaaactccatttccacccctcccagttcccaactattttgtccgcccacagcggggcatttttcttcctgttatgtttttaatcaaacatcctgccaactccatgtgacaaaccgtcatcttcggctacttt

SEQ ID NO: 2 - DNA, 21 bp, Artificial sequence
  ITR forward primer
ggaacccctagtgatggagtt

SEQ ID NO: 3 - DNA, 16 bp, Artificial sequence
  ITR reverse primer
cggcctcagtgagcga

SEQ ID NO: 4 - DNA, 2208 bp, Artificial sequence
  Cap gene sequence
acggctgccgacggttatctacccgattggctcgaggacactctctctgaaggaataagacagtggtggaagctcaaacccggcccaccaccaccaaagcccgcagagcggcataaggacgacagcaggggccttgtgcttcccgggtacaagtacctcggacccttcaacggactggacaagggagagccggtgaacgaggcagacgccgctgccctcgagcacgacaaagcctacgaccggcagctcgacagcggagacaacccttacctcaagtacaaccacgccgacgcggagttccaggagcgccttaaagaagatacgtcttttgggggcaacctcggacgagcagtcttccaggcgaaaaagagggttcttgaacctctgggcctggttgaggaacctgttaagacggctccgggaaaaaagaggccggtagagcactctcctgtggagccagactcctcctcgggaaccggaaaggcgggccagcagcctgcaagaaaaagattgaattttggtcagactggagacgcagactcagtacctgacccccagcctctcggacagccaccagcagccccctctggtctgggaactaatacgatggctacaggcagtggcgcaccaatggcagacaataacgagggcgccgacggagtgggtaattcctcgggaaattggcattgcgattccacatggatgggcgacagagtcatcaccaccagcacccgaacctgggccctgcccacctacaacaaccacctctacaaacaaatttccagccaatcaggagcctcgaacgacaatcactactttggctacagcaccccttgggggtattttgacttcaacagattccactgccacttttcaccacgtgactggcaaagactcatcaacaacaactggggattccgacccaagagactcaacttcaagctctttaacattcaagtcaaagaggtcacgcagaatgacggtacgacgacgattgccaataaccttaccagcacggttcaggtgtttactgactcggagtaccagctcccgtacgtcctcggctcggcgcatcaaggatgcctcccgccgttcccagcagacgtcttcatggtgccacagtatggatacctcaccctgaacaacgggagtcaggcagtaggacgctcttcattttactgcctggagtactttccttctcagatgctgcgtaccggaaacaactttaccttcagctacacttttgaggacgttcctttccacagcagctacgctcacagccagagtctggaccgtctcatgaatcctctcatcgaccagtacctgtattacttgagcagaacaaacactccaagtggaaccaccacgcagtcaaggcttcagttttctcaggccggagcgagtgacattcgggaccagtctaggaactggcttcctggaccctgttaccgccagcagcgagtatcaaagacatctgcggataacaacaacagtgaatactcgtggactggagctaccaagtaccacctcaatggcagagactctctggtgaatccgggcccggcgatggcaagccacaaggacgatgaagaaaagttttttcctcagagcggggttctcatctttgggaagcaaggctcagagaaaacaaatgtggacattgaaaaggtcatgattacagacgaagaggaaatcaggacaaccaatcccgtggctacggagcagtatggttctgtatctaccaacctccagagaggcaacagacaagcagctaccgcagatgtcaacacacaaggcgttcttccaggcatggtctggcaggacagagatgtgtaccttcaggggcccatctgggcaaagattccacacacggacggacattttcacccctctcccctcatgggtggattcggacttaaacaccctcctccacagattctcatcaagaacaccccggtacctgcgaatccttcgaccaccttcagtgcggcaaagtttgcttccttcatcacacagtactccacgggacaggtcagcgtggagatcgagtgggagctgcagaaggaaaacagcaaacgctggaatcccgaaattcagtacacttccaactacaacaagtctgttaatgtggactttactgtggacactaatggcgtgtattcagagcctcgccccattggcaccagatacctgactcgtaatctgtaa

SEQ ID NO: 5 - DNA, 1866 bp, Artificial sequence
  Rep gene sequence
ctggcggggttttacgagattgtgattaaggtccccagcgaccttgacgagcatctgcccggcatttctgacagctttgtgaactgggtggccgagaaggagtgggagttgccgccagattctgacttggatctgaatctgattgagcaggcacccctgaccgtggccgagaagctgcagcgcgactttctgacggagtggcgccgtgtgagtaaggccccggaggcccttttctttgtgcaatttgagaagggagagagctacttccacttacacgtgctcgtggaaaccaccggggtgaaatccttagttttgggacgtttcctgagtcagattcgcgaaaaactgattcagagaatttaccgcgggatcgagccgactttgccaaactggttcgcggtcacaaagaccagaaacggcgccggaggcgggaacaaggtggtggacgagtgctacatccccaattacttgctccccaaaacccagcctgagctccagtgggcgtggactaatttagaacagtatttaagcgcctgtttgaatctcacggagcgtaaacggttggtggcgcagcatctgacgcacgtgtcgcagacgcaggagcagaacaaagagaatcagaatcccaattctgacgcgccggtgatcagatcaaaaacttcagccaggtacatggagctggtcgggtggctcgtggacaaggggattacctcggagaagcagtggatacaggaggaccaggcctcatacatctccttcaatgcggcctccaactcgcggtcccaaatcaaggctgccttggacaatgcgggaaagattatgagcctgactaaaaccgcccccgactacctggtgggccagcagcccgtggaggacatttccagcaatcggatttataaaattttggaactaaacgggtacgatccccaatatgcggcttccgtctttctgggatgggccacgaaaaagttcggcaagaggaacaccatctggctgtttgggcctgcaactaccgggaagaccaacatcgcggaggccatagcccacactgtgcccttctacgggtgcgtaaactggaccaatgagaactttcccttcaacgactgtgtggacaagatggtgatctggtgggaggaggggaagatgaccgccaaggtcgtggagtcggccaaagccattctcggaggaagcaaggtgcgcgtggaccagaaatgcaagtcctcggcccagatagacccgactcccgtgatcgtcacctccaacaccaacatgtgcgccgtgattgacgggaactcaacgaccttcgaacaccagcagccgttgcaagaccggatgttcaaatttgaactcacccgccgtctggatcatgactttgggaaggtcaccaagcaggaagtcaaagactttttccggtgggcaaaggatcacgtggttgaggtggagcatgaattctacgtcaaaaagggtggagccaagaaaagacccgcccccagtgacgcagatataagtgagcccaaacgggtgcgcgagtcagttgcgcagccatcgacgtcagacgcggaagcatcgatcaactacgcagacaggtaccaaaacaaatgttctcgtcacgtgggcatgaatctgatgctgtttccctgcagacaatgcgagagaatgaatcagaattcaaatatctgcttcactcacggacagaaagactgtttagagtgctttcccgtgtcagaatctcaacccgtttctgtcgtcaaaaaggcgtatcagaaactgtgctacattcatcatatcatgggaaaggtgccagacgcttgcactgcctgcgatctggtcaatgtggatttggatgactgcatctttgaacaataa

SEQ ID NO: 6 - DNA, 1388 bp, Artificial sequence
  Nucleotide sequence of hr1-p6.9-p10 promoter
atcgatgttgaccccaacaaaagatttataattaatcataatcacgaacaacaacaagtcaatgaaacaaataaacaagttgtcgataaaacattcataaatgacacagcaacatacaattcttgcataataaaaatttaaatgacatcatatttgagaataacaaatgacattatccctcgattgtgttttacaagtagaattctacccgtaaagcgagtttagttttgaaaaacaaatgacatcatttgtataatgacatcatcccctgattgtgttttacaagtagaattctatccgtaaagcgagttcagttttgaaaacaaatgagtcatacctaaacacgttaataatcttctgatatcagcttatgactcaagttatgagccgtgtgcaaaacatgagataagtttatgacatcatccactgatcgtgcgttacaagtagaattctactcgtaaagccagttcggttatgagccgtgtgcaaaacatgacatcagcttatgactcatacttgattgtgttttacgcgtagaattctactcgtaaagcgagttcggttatgagccgtgtgcaaaacatgacatcagcttatgagtcataattaatcgtgcgttacaagtagaattctactcgtaaagcgagttgaaggatcatatttagttgcgtttatgagataagattgaaagcacgtgtaaaatgtttcccgcgcgttggcacaactatttacaatgcggccaagttataaaagattctaatctgatatgttttaaaacacctttgcggcccgagttgtttgcgtacgtgactagcgaagaagatgtgtggaccgcagaacagatagtaaaacaaaaccctagtattggagcaataatcgatgacgtcgctgacgtagcgctttgaattccgcgcgcttcggaccgggatcgtgaccaaattccgttttgcgacgatgcagagtttttgaacaggctgctcaaacacatagatccgtacccgctcagtcggatgtattacaatgcagccaataccatgttttacacgactatggaaaactatgccgtgtccaattgcaagttcaacattgaggattacaataacatatttaaggtgatggaaaatattaggaaacacagcaacaaaaattcaaacgaccaagacgagttaaacatatatttgggagttcagtcgtcgaatgcaaagcgtaaaaaatattaataaggtaaaaattacagctacataaattacacaatttaaactgcagtctggagatacggacctttaattcaacccaacacaatatattatagttaaataagaattattatcaaatcatttgtatattaattaaaatactatactgtaaattacattttatttacaatc

SEQ ID NO: 7 - DNA, 2202 bp, Artificial sequence
  Nucleotide sequence of pH-Acie01
aacttgtttattgcagcttataatggttacaaataaagcaatagcatcacaaatttcacaaataaagcatttttttcactgcattctagttgtggtttgtccaaactcatcaatgtatcttatcatgtctggatctgatcactgcttgagcctaggagatccgatcatggagataattaaaatgataaccatctcgcaaataaataagtattttactgttttcgtaacagttttgtaataaaaaaacctataaatattccggattattcataccgtcccaccatcgggcgcatgatccgtacatccagccacgtcctgaacgtccaagaaaacatcatgacttccaactgtgcttccagcccctactcctgtgaggccacttcagcctgcgctgaggcccagcaactgcaggtggacacaggtggcgataagatcgtgaacaaccaggtcaccatgactcaaatcaacttcaacgcttcctacacctctgccagcactccctctcgtgctagcttcgacaactcatactcggagttctgcgacaagcaacctaacgattacttgtcttactacaaccacccaaccccggacggagctgatactgtcatctccgactctgaaaccgctgccgctagcaacttcctcgcctcagttaactcgctcactgacaacgatttggtggagtgtctgctcaagaccactgacaacctggaggaagctgtgtcctctgcctactacagcgagtcactcgaacagccagtggtcgaacaaccctctcctagctcagcttaccacgccgagtccttcgaacactctgctggtgtcaaccagccgtcggccacaggcaccaagaggaagttggacgagtacctggataactcccagggagttgtgggtcaattcaacaagatcaagttgagacctaagtacaagaagagcaccatccagtcatgcgctacactggaacaaaccatcaaccacaacactaacatctgtacagtggcttccacccaggagatcactcactacttcacaaacgacttcgccccctacctgatgaggttcgacgataacgactacaactcgaacagattctccgatcacatgtctgaaaccggttactacatgttcgtcgttaagaagtccgaggtgaagcctttcgaaatcatcttcgccaagtacgtctctaacgtggtctacgagtacacaaacaactactacatggttgacaaccgtgtgttcgttgtgaccttcgataagatccgcttcatgatcagctacaacctggttaaggagactggcatcgaaatcccacactcacaggacgtctgcaacgatgagaccgccgctcaaaactgcaagaagtgtcacttcgtggacgtccaccacacattcaaggccgctctgacctcctacttcaacctcgatatgtactacgctcagacaaccttcgtgaccttgctgcaatcactcggcgagcgtaagtgtggattcctcttgtcgaagttgtacgagatgtaccaggacaagaacctcttcactttgcccatcatgctgagccgcaaggaatcaaacgagatcgaaaccgcctctaacaacttcttcgtctcgccatacgtttcccagatcctcaagtactcggagtccgtccaattcccggacaaccctcccaacaagtacgtcgttgataacctgaacctcatcgtgaacaagaagagcactctgacatacaagtactcgtccgtcgctaacctgctcttcaacaactacaagtaccacgacaacatcgcttctaacaacaacgccgagaacctcaagaaggtcaagaaggaagacggaagcatgcacatcgttgagcagtacttgactcaaaacgtcgataacgttaagggtcacaacttcatcgtgttgtccttcaagaacgaggaaaggctgaccatcgctaagaagaacaaggagttctactggatctctggcgaaatcaaggacgttgatgtgagccaggtcatccaaaagtacaacagattcaagcaccacatgttcgtgatcggcaaggtcaaccgtcgcgagtcaactacactgcacaacaacttgctgaagctcttggccttgatcctgcagggactggtgccactctccgacgccatcacattcgccgagcaaaagctcaactgcaagtacaagaagttcgagttcaactaa

SEQ ID NO: 8 - DNA, 11248 bp, Artificial sequence
  Nucleotide sequence of pFBd-Cap-ITR-Rep
ttctctgtcacagaatgaaaatttttctgtcatctcttcgttattaatgtttgtaattgactgaatatcaacgcttatttgcagcctgaatggcgaatgggacgcgccctgtagcggcgcattaagcgcggcgggtgtggtggttacgcgcagcgtgaccgctacacttgccagcgccctagcgcccgctcctttcgctttcttcccttcctttctcgccacgttcgccggctttccccgtcaagctctaaatcgggggctccctttagggttccgatttagtgctttacggcacctcgaccccaaaaaacttgattagggtgatggttcacgtagtgggccatcgccctgatagacggtttttcgccctttgacgttggagtccacgttctttaatagtggactcttgttccaaactggaacaacactcaaccctatctcggtctattcttttgatttataagggattttgccgatttcggcctattggttaaaaaatgagctgatttaacaaaaatttaacgcgaattttaacaaaatattaacgtttacaatttcaggtggcacttttcggggaaatgtgcgcggaacccctatttgtttatttttctaaatacattcaaatatgtatccgctcatgagacaataaccctgataaatgcttcaataatattgaaaaaggaagagtatgagtattcaacatttccgtgtcgcccttattcccttttttgcggcattttgccttcctgtttttgctcacccagaaacgctggtgaaagtaaaagatgctgaagatcagttgggtgcacgagtgggttacatcgaactggatctcaacagcggtaagatccttgagagttttcgccccgaagaacgttttccaatgatgagcacttttaaagttctgctatgtggcgcggtattatcccgtattgacgccgggcaagagcaactcggtcgccgcatacactattctcagaatgacttggttgagtactcaccagtcacagaaaagcatcttacggatggcatgacagtaagagaattatgcagtgctgccataaccatgagtgataacactgcggccaacttacttctgacaacgatcggaggaccgaaggagctaaccgcttttttgcacaacatgggggatcatgtaactcgccttgatcgttgggaaccggagctgaatgaagccataccaaacgacgagcgtgacaccacgatgcctgtagcaatggcaacaacgttgcgcaaactattaactggcgaactacttactctagcttcccggcaacaattaatagactggatggaggcggataaagttgcaggaccacttctgcgctcggcccttccggctggctggtttattgctgataaatctggagccggtgagcgtgggtctcgcggtatcattgcagcactggggccagatggtaagccctcccgtatcgtagttatctacacgacggggagtcaggcaactatggatgaacgaaatagacagatcgctgagataggtgcctcactgattaagcattggtaactgtcagaccaagtttactcatatatactttagattgatttaaaacttcatttttaatttaaaaggatctaggtgaagatcctttttgataatctcatgaccaaaatcccttaacgtgagttttcgttccactgagcgtcagaccccgtagaaaagatcaaaggatcttcttgagatcctttttttctgcgcgtaatctgctgcttgcaaacaaaaaaaccaccgctaccagcggtggtttgtttgccggatcaagagctaccaactctttttccgaaggtaactggcttcagcagagcgcagataccaaatactgtccttctagtgtagccgtagttaggccaccacttcaagaactctgtagcaccgcctacatacctcgctctgctaatcctgttaccagtggctgctgccagtggcgataagtcgtgtcttaccgggttggactcaagacgatagttaccggataaggcgcagcggtcgggctgaacggggggttcgtgcacacagcccagcttggagcgaacgacctacaccgaactgagatacctacagcgtgagcattgagaaagcgccacgcttcccgaagggagaaaggcggacaggtatccggtaagcggcagggtcggaacaggagagcgcacgagggagcttccagggggaaacgcctggtatctttatagtcctgtcgggtttcgccacctctgacttgagcgtcgatttttgtgatgctcgtcaggggggcggagcctatggaaaaacgccagcaacgcggcctttttacggttcctggccttttgctggccttttgctcacatgttctttcctgcgttatcccctgattctgtggataaccgtattaccgcctttgagtgagctgataccgctcgccgcagccgaacgaccgagcgcagcgagtcagtgagcgaggaagcggaagagcgcctgatgcggtattttctccttacgcatctgtgcggtatttcacaccgcagaccagccgcgtaacctggcaaaatcggttacggttgagtaataaatggatgccctgcgtaagcgggtgtgggcggacaataaagtcttaaactgaacaaaatagatctaaactatgacaataaagtcttaaactagacagaatagttgtaaactgaaatcagtccagttatgctgtgaaaaagcatactggacttttgttatggctaaagcaaactcttcattttctgaagtgcaaattgcccgtcgtattaaagaggggcgtggccaagggcatggtaaagactatattcgcggcgttgtgacaatttaccgaacaactccgcggccgggaagccgatctcggcttgaacgaattgttaggtggcggtacttgggtcgatatcaaagtgcatcacttcttcccgtatgcccaactttgtatagagagccactgcgggatcgtcaccgtaatctgcttgcacgtagatcacataagcaccaagcgcgttggcctcatgcttgaggagattgatgagcgcggtggcaatgccctgcctccggtgctcgccggagactgcgagatcatagatatagatctcactacgcggctgctcaaacctgggcagaacgtaagccgcgagagcgccaacaaccgcttcttggtcgaaggcagcaagcgcgatgaatgtcttactacggagcaagttcccgaggtaatcggagtccggctgatgttgggagtaggtggctacgtctccgaactcacgaccgaaaagatcaagagcagcccgcatggatttgacttggtcagggccgagcctacatgtgcgaatgatgcccatacttgagccacctaactttgttttagggcgactgccctgctgcgtaacatcgttgctgctgcgtaacatcgttgctgctccataacatcaaacatcgacccacggcgtaacgcgcttgctgcttggatgcccgaggcatagactgtacaaaaaaacagtcataacaagccatgaaaaccgccactgcgccgttaccaccgctgcgttcggtcaaggttctggaccagttgcgtgagcgcatacgctacttgcattacagtttacgaaccgaacaggcttatgtcaactgggttcgtgccttcatccgtttccacggtgtgcgtcacccggcaaccttgggcagcagcgaagtcgaggcatttctgtcctggctggcgaacgagcgcaaggtttcggtctccacgcatcgtcaggcattggcggccttgctgttcttctacggcaaggtgctgtgcacggatctgccctggcttcaggagatcggtagacctcggccgtcgcggcgcttgccggtggtgctgaccccggatgaagtggttcgcatcctcggttttctggaaggcgagcatcgtttgttcgcccaggactctagctatagttctagtggttggcctacgtacccgtagtggctatggcagggcttgccgccccgacgttggctgcgagccctgggccttcacccgaacttgggggttggggtggggaaaaggaagaaacgcgggcgtattggtcccaatggggtctcggtggggtatcgacagagtgccagccctgggaccgaaccccgcgtttatgaacaaacgacccaacacccgtgcgttttattctgtctttttattgccgtcatagcgcgggttccttccggtattgtctccttccgtgtttcagttagcctcccccatctcccggtaccgcatgcttacagattacgagtcaggtatctggtgccaatggggcgaggctctgaatacacgccattagtgtccacagtaaagtccacattaacagacttgttgtagttggaagtgtactgaatttcgggattccagcgtttgctgttttccttctgcagctcccactcgatctccacgctgacctgtcccgtggagtactgtgtgatgaaggaagcaaactttgccgcactgaaggtggtcgaaggattcgcaggtaccggggtgttcttgatgagaatctgtggaggagggtgtttaagtccgaatccacccatgaggggagaggggtgaaaatgtccgtccgtgtgtggaatctttgcccagatgggcccctgaaggtacacatctctgtcctgccagaccatgcctggaagaacgccttgtgtgttgacatctgcggtagctgcttgtctgttgcctctctggaggttggtagatacagaaccatactgctccgtagccacgggattggttgtcctgatttcctcttcgtctgtaatcatgaccttttcaatgtccacatttgttttctctgagccttgcttcccaaagatgagaaccccgctctgaggaaaaaacttttcttcatcgtccttgtggcttgccatcgccgggcccggattcaccagagagtctctgccattgaggtggtacttggtagctccagtccacgagtattcactgttgttgttatccgcagatgtctttgatactcgctgctggcggtaacagggtccaggaagccagttcctagactggtcccgaatgtcactcgctccggcctgagaaaactgaagccttgactgcgtggtggttccacttggagtgtttgttctgctcaagtaatacaggtactggtcgatgagaggattcatgagacggtccagactctggctgtgagcgtagctgctgtggaaaggaacgtcctcaaaagtgtagctgaaggtaaagttgtttccggtacgcagcatctgagaaggaaagtactccaggcagtaaaatgaagagcgtcctactgcctgactcccgttgttcagggtgaggtatccatactgtggcaccatgaagacgtctgctgggaacggcgggaggcatccttgatgcgccgagccgaggacgtacgggagctggtactccgagtcagtaaacacctgaaccgtgctggtaaggttattggcaatcgtcgtcgtaccgtcattctgcgtgacctctttgacttgaatgttaaagagcttgaagttgagtctcttgggtcggaatccccagttgttgttgatgagtctttgccagtcacgtggtgaaaagtggcagtggaatctgttgaagtcaaaatacccccaaggggtgctgtagccaaagtagtgattgtcgttcgaggctcctgattggctggaaatttgtttgtagaggtggttgttgtaggtgggcagggcccaggttcgggtgctggtggtgatgactctgtcgcccatccatgtggaatcgcaatgccaatttcccgaggaattacccactccgtcggcgccctcgttattgtctgccattggtgcgccactgcctgtagccatcgtattagttcccagaccagagggggctgctggtggctgtccgagaggctgggggtcaggtactgagtctgcgtctccagtctgaccaaaattcaatctttttcttgcaggctgctggcccgcctttccggttcccgaggaggagtctggctccacaggagagtgctctaccggcctcttttttcccggagccgtcttaacaggttcctcaaccaggcccagaggttcaagaaccctctttttcgcctggaagactgctcgtccgaggttgcccccaaaagacgtatcttctttaaggcgctcctggaactccgcgtcggcgtggttgtacttgaggtaagggttgtctccgctgtcgagctgccggtcgtaggctttgtcgtgctcgagggcagcggcgtctgcctcgttcaccggctctcccttgtccagtccgttgaagggtccgaggtacttgtacccgggaagcacaaggcccctgctgtcgtccttatgccgctctgcgggctttggtggtggtgggccgggtttgagcttccaccactgtcttattccttcagagagagtgtcctcgagccaatcgggtagataaccgtcggcagccgtggcggcgctagcaccatggctcgagatcccgggtgatcaagtcttcgtcgagtgattgtaaataaaatgtaatttacagtatagtattttaattaatatacaaatgatttgataataattcttatttaactataatatattgtgttgggttgaattaaaggtccgtatacgccgctacagggcgcgtactatggttgctttgacgtatgcggtgtgaaataccgcacagatgcgtaaggagaaaataccgcatcaggcgcccctgcaggcagctgcgcgctcgctcgctcactgaggccgcccgggcaaagcccgggcgtcgggcgacctttggtcgcccggcctcagtgagcgagcgagcgcgcagagagggagtggccaactccatcactaggggttcctacgcgttagttattaatagtaatcaattacggggtcattagttcatagcccatatatggagttccgcgttacataacttacggtaaatggcccgcctggctgaccgcccaacgacccccgcccattgacgtcaataatgacgtatgttcccatagtaacgccaatagggactttccattgacgtcaatgggtggagtatttacggtaaactgcccacttggcagtacatcaagtgtatcatatgccaagtacgccccctattgacgtcaatgacggtaaatggcccgcctggcattatgcccagtacatgaccttatgggactttcctacttggcagtacatctacgtattagtcatcgctattaccatggtgatgcggttttggcagtacatcaatgggcgtggatagcggtttgactcacggggatttccaagtctccaccccattgacgtcaatgggagtttgttttggcaccaaaatcaacgggactttccaaaatgtcgtaacaactccgccccattgacgcaaatgggcggtaggcgtgtacggtgggaggtctatataagcagagctggtttagtgaaccgtcagatccgctagcgctaccggtcgccaccatggtgagcaagggcgaggagctgttcaccggggtggtgcccatcctggtcgagctggacggcgacgtaaacggccacaagttcagcgtgtccggcgagggcgagggcgatgccacctacggcaagctgaccctgaagttcatctgcaccaccggcaagctgcccgtgccctggcccaccctcgtgaccaccctgacctacggcgtgcagtgcttcagccgctaccccgaccacatgaagcagcacgacttcttcaagtccgccatgcccgaaggctacgtccaggagcgcaccatcttcttcaaggacgacggcaactacaagacccgcgccgaggtgaagttcgagggcgacaccctggtgaaccgcatcgagctgaagggcatcgacttcaaggaggacggcaacatcctggggcacaagctggagtacaactacaacagccacaacgtctatatcatggccgacaagcagaagaacggcatcaaggtgaacttcaagatccgccacaacatcgaggacggcagcgtgcagctcgccgaccactaccagcagaacacccccatcggcgacggccccgtgctgctgcccgacaaccactacctgagcacccagtccgccctgagcaaagaccccaacgagaagcgcgatcacatggtcctgctggagttcgtgaccgccgccgggatcactctcggcatggacgagctgtacaagtaggtcgacgtttatttgtgaaatttgtgatgctattgctttatttgtaaccatctagctttatttgtgaaatttgtgatgctattgctttatttgtaaccattataagctgcaataaacaagttaacaacaacaattgcattcattttatgtttcaggttcagggggagatgtgggaggttttttaaagtttaaacaggaacccctagtgatggagttggccactccctctctgcgcgctcgctcgctcactgaggccgggcgaccaaaggtcgcccgacgcccgggcggcctcagtgagcgagcgagcgcgcagctgcctgcaggacatgtgagcaaaaggccagcaaaaggccaggaaccgtaaaaaggccgcgttgctggcgtttttccataggctccgcccccctgacgagcatcacaaaaatcgacgctcgcggccgctctagagatcatggagataattaaaatgataaccatctcgcaaataaataagtattttactgttttcgtaacagttttgtaataaaaaaacctataaatattccggattattcataccgtcccaccatcgggcgcggatccgccgccctggcggggttttacgagattgtgattaaggtccccagcgaccttgacgagcatctgcccggcatttctgacagctttgtgaactgggtggccgagaaggagtgggagttgccgccagattctgacttggatctgaatctgattgagcaggcacccctgaccgtggccgagaagctgcagcgcgactttctgacggagtggcgccgtgtgagtaaggccccggaggcccttttctttgtgcaatttgagaagggagagagctacttccacttacacgtgctcgtggaaaccaccggggtgaaatccttagttttgggacgtttcctgagtcagattcgcgaaaaactgattcagagaatttaccgcgggatcgagccgactttgccaaactggttcgcggtcacaaagaccagaaacggcgccggaggcgggaacaaggtggtggacgagtgctacatccccaattacttgctccccaaaacccagcctgagctccagtgggcgtggactaatttagaacagtatttaagcgcctgtttgaatctcacggagcgtaaacggttggtggcgcagcatctgacgcacgtgtcgcagacgcaggagcagaacaaagagaatcagaatcccaattctgacgcgccggtgatcagatcaaaaacttcagccaggtacatggagctggtcgggtggctcgtggacaaggggattacctcggagaagcagtggatacaggaggaccaggcctcatacatctccttcaatgcggcctccaactcgcggtcccaaatcaaggctgccttggacaatgcgggaaagattatgagcctgactaaaaccgcccccgactacctggtgggccagcagcccgtggaggacatttccagcaatcggatttataaaattttggaactaaacgggtacgatccccaatatgcggcttccgtctttctgggatgggccacgaaaaagttcggcaagaggaacaccatctggctgtttgggcctgcaactaccgggaagaccaacatcgcggaggccatagcccacactgtgcccttctacgggtgcgtaaactggaccaatgagaactttcccttcaacgactgtgtggacaagatggtgatctggtgggaggaggggaagatgaccgccaaggtcgtggagtcggccaaagccattctcggaggaagcaaggtgcgcgtggaccagaaatgcaagtcctcggcccagatagacccgactcccgtgatcgtcacctccaacaccaacatgtgcgccgtgattgacgggaactcaacgaccttcgaacaccagcagccgttgcaagaccggatgttcaaatttgaactcacccgccgtctggatcatgactttgggaaggtcaccaagcaggaagtcaaagactttttccggtgggcaaaggatcacgtggttgaggtggagcatgaattctacgtcaaaaagggtggagccaagaaaagacccgcccccagtgacgcagatataagtgagcccaaacgggtgcgcgagtcagttgcgcagccatcgacgtcagacgcggaagcatcgatcaactacgcagacaggtaccaaaacaaatgttctcgtcacgtgggcatgaatctgatgctgtttccctgcagacaatgcgagagaatgaatcagaattcaaatatctgcttcactcacggacagaaagactgtttagagtgctttcccgtgtcagaatctcaacccgtttctgtcgtcaaaaaggcgtatcagaaactgtgctacattcatcatatcatgggaaaggtgccagacgcttgcactgcctgcgatctggtcaatgtggatttggatgactgcatctttgaacaataatctagagcctgcagtctcgacaagcttgtcgagaagtactagaggatcataatcagccataccacatttgtagaggttttacttgctttaaaaaacctcccacacctccccctgaacctgaaacataaaatgaatgcaattgttgttgttaacttgtttattgcagcttataatggttacaaataaagcaatagcatcacaaatttcacaaataaagcatttttttcactgcattctagttgtggtttgtccaaactcatcaatgtatcttatcatgtctggatctgatcactgcttgagcctaggagatccgaaccagataagtgaaatctagttccaaactattttgtcatttttaattttcgtattagcttacgacgctacacccagttcccatctattttgtcactcttccctaaataatccttaaaaactccatttccacccctcccagttcccaactattttgtccgcccacagcggggcatttttcttcctgttatgtttttaatcaaacatcctgccaactccatgtgacaaaccgtcatcttcggctacttt

SEQ ID NO: 9 - DNA, 14777 bp, Artificial sequence
  Nucleotide sequence of pFBd-IE-hr1Cap-ITR-Rep
ttctctgtcacagaatgaaaatttttctgtcatctcttcgttattaatgtttgtaattgactgaatatcaacgcttatttgcagcctgaatggcgaatgggacgcgccctgtagcggcgcattaagcgcggcgggtgtggtggttacgcgcagcgtgaccgctacacttgccagcgccctagcgcccgctcctttcgctttcttcccttcctttctcgccacgttcgccggctttccccgtcaagctctaaatcgggggctccctttagggttccgatttagtgctttacggcacctcgaccccaaaaaacttgattagggtgatggttcacgtagtgggccatcgccctgatagacggtttttcgccctttgacgttggagtccacgttctttaatagtggactcttgttccaaactggaacaacactcaaccctatctcggtctattcttttgatttataagggattttgccgatttcggcctattggttaaaaaatgagctgatttaacaaaaatttaacgcgaattttaacaaaatattaacgtttacaatttcaggtggcacttttcggggaaatgtgcgcggaacccctatttgtttatttttctaaatacattcaaatatgtatccgctcatgagacaataaccctgataaatgcttcaataatattgaaaaaggaagagtatgagtattcaacatttccgtgtcgcccttattcccttttttgcggcattttgccttcctgtttttgctcacccagaaacgctggtgaaagtaaaagatgctgaagatcagttgggtgcacgagtgggttacatcgaactggatctcaacagcggtaagatccttgagagttttcgccccgaagaacgttttccaatgatgagcacttttaaagttctgctatgtggcgcggtattatcccgtattgacgccgggcaagagcaactcggtcgccgcatacactattctcagaatgacttggttgagtactcaccagtcacagaaaagcatcttacggatggcatgacagtaagagaattatgcagtgctgccataaccatgagtgataacactgcggccaacttacttctgacaacgatcggaggaccgaaggagctaaccgcttttttgcacaacatgggggatcatgtaactcgccttgatcgttgggaaccggagctgaatgaagccataccaaacgacgagcgtgacaccacgatgcctgtagcaatggcaacaacgttgcgcaaactattaactggcgaactacttactctagcttcccggcaacaattaatagactggatggaggcggataaagttgcaggaccacttctgcgctcggcccttccggctggctggtttattgctgataaatctggagccggtgagcgtgggtctcgcggtatcattgcagcactggggccagatggtaagccctcccgtatcgtagttatctacacgacggggagtcaggcaactatggatgaacgaaatagacagatcgctgagataggtgcctcactgattaagcattggtaactgtcagaccaagtttactcatatatactttagattgatttaaaacttcatttttaatttaaaaggatctaggtgaagatcctttttgataatctcatgaccaaaatcccttaacgtgagttttcgttccactgagcgtcagaccccgtagaaaagatcaaaggatcttcttgagatcctttttttctgcgcgtaatctgctgcttgcaaacaaaaaaaccaccgctaccagcggtggtttgtttgccggatcaagagctaccaactctttttccgaaggtaactggcttcagcagagcgcagataccaaatactgtccttctagtgtagccgtagttaggccaccacttcaagaactctgtagcaccgcctacatacctcgctctgctaatcctgttaccagtggctgctgccagtggcgataagtcgtgtcttaccgggttggactcaagacgatagttaccggataaggcgcagcggtcgggctgaacggggggttcgtgcacacagcccagcttggagcgaacgacctacaccgaactgagatacctacagcgtgagcattgagaaagcgccacgcttcccgaagggagaaaggcggacaggtatccggtaagcggcagggtcggaacaggagagcgcacgagggagcttccagggggaaacgcctggtatctttatagtcctgtcgggtttcgccacctctgacttgagcgtcgatttttgtgatgctcgtcaggggggcggagcctatggaaaaacgccagcaacgcggcctttttacggttcctggccttttgctggccttttgctcacatgttctttcctgcgttatcccctgattctgtggataaccgtattaccgcctttgagtgagctgataccgctcgccgcagccgaacgaccgagcgcagcgagtcagtgagcgaggaagcggaagagcgcctgatgcggtattttctccttacgcatctgtgcggtatttcacaccgcagaccagccgcgtaacctggcaaaatcggttacggttgagtaataaatggatgccctgcgtaagcgggtgtgggcggacaataaagtcttaaactgaacaaaatagatctaaactatgacaataaagtcttaaactagacagaatagttgtaaactgaaatcagtccagttatgctgtgaaaaagcatactggacttttgttatggctaaagcaaactcttcattttctgaagtgcaaattgcccgtcgtattaaagaggggcgtggccaagggcatggtaaagactatattcgcggcgttgtgacaatttaccgaacaactccgcggccgggaagccgatctcggcttgaacgaattgttaggtggcggtacttgggtcgatatcaaagtgcatcacttcttcccgtatgcccaactttgtatagagagccactgcgggatcgtcaccgtaatctgcttgcacgtagatcacataagcaccaagcgcgttggcctcatgcttgaggagattgatgagcgcggtggcaatgccctgcctccggtgctcgccggagactgcgagatcatagatatagatctcactacgcggctgctcaaacctgggcagaacgtaagccgcgagagcgccaacaaccgcttcttggtcgaaggcagcaagcgcgatgaatgtcttactacggagcaagttcccgaggtaatcggagtccggctgatgttgggagtaggtggctacgtctccgaactcacgaccgaaaagatcaagagcagcccgcatggatttgacttggtcagggccgagcctacatgtgcgaatgatgcccatacttgagccacctaactttgttttagggcgactgccctgctgcgtaacatcgttgctgctgcgtaacatcgttgctgctccataacatcaaacatcgacccacggcgtaacgcgcttgctgcttggatgcccgaggcatagactgtacaaaaaaacagtcataacaagccatgaaaaccgccactgcgccgttaccaccgctgcgttcggtcaaggttctggaccagttgcgtgagcgcatacgctacttgcattacagtttacgaaccgaacaggcttatgtcaactgggttcgtgccttcatccgtttccacggtgtgcgtcacccggcaaccttgggcagcagcgaagtcgaggcatttctgtcctggctggcgaacgagcgcaaggtttcggtctccacgcatcgtcaggcattggcggccttgctgttcttctacggcaaggtgctgtgcacggatctgccctggcttcaggagatcggtagacctcggccgtcgcggcgcttgccggtggtgctgaccccggatgaagtggttcgcatcctcggttttctggaaggcgagcatcgtttgttcgcccaggactctagctatagttctagtggttggcctacgtacccgtagtggctatggcagggcttgccgccccgacgttggctgcgagccctgggccttcacccgaacttgggggttggggtggggaaaaggaagaaacgcgggcgtattggtcccaatggggtctcggtggggtatcgacagagtgccagccctgggaccgaaccccgcgtttatgaacaaacgacccaacacccgtgcgttttattctgtctttttattgccgtcatagcgcgggttccttccggtattgtctccttccgtgtttcagttagcctcccccatctcccggtaccgcatgccttagttgaactcgaacttcttgtacttgcagttgagcttttgctcggcgaatgtgatggcgtcggagagtggcaccagtccctgcaggatcaaggccaagagcttcagcaagttgttgtgcagtgtagttgactcgcgacggttgaccttgccgatcacgaacatgtggtgcttgaatctgttgtacttttggatgacctggctcacatcaacgtccttgatttcgccagagatccagtagaactccttgttcttcttagcgatggtcagcctttcctcgttcttgaaggacaacacgatgaagttgtgacccttaacgttatcgacgttttgagtcaagtactgctcaacgatgtgcatgcttccgtcttccttcttgaccttcttgaggttctcggcgttgttgttagaagcgatgttgtcgtggtacttgtagttgttgaagagcaggttagcgacggacgagtacttgtatgtcagagtgctcttcttgttcacgatgaggttcaggttatcaacgacgtacttgttgggagggttgtccgggaattggacggactccgagtacttgaggatctgggaaacgtatggcgagacgaagaagttgttagaggcggtttcgatctcgtttgattccttgcggctcagcatgatgggcaaagtgaagaggttcttgtcctggtacatctcgtacaacttcgacaagaggaatccacacttacgctcgccgagtgattgcagcaaggtcacgaaggttgtctgagcgtagtacatatcgaggttgaagtaggaggtcagagcggccttgaatgtgtggtggacgtccacgaagtgacacttcttgcagttttgagcggcggtctcatcgttgcagacgtcctgtgagtgtgggatttcgatgccagtctccttaaccaggttgtagctgatcatgaagcggatcttatcgaaggtcacaacgaacacacggttgtcaaccatgtagtagttgtttgtgtactcgtagaccacgttagagacgtacttggcgaagatgatttcgaaaggcttcacctcggacttcttaacgacgaacatgtagtaaccggtttcagacatgtgatcggagaatctgttcgagttgtagtcgttatcgtcgaacctcatcaggtagggggcgaagtcgtttgtgaagtagtgagtgatctcctgggtggaagccactgtacagatgttagtgttgtggttgatggtttgttccagtgtagcgcatgactggatggtgctcttcttgtacttaggtctcaacttgatcttgttgaattgacccacaactccctgggagttatccaggtactcgtccaacttcctcttggtgcctgtggccgacggctggttgacaccagcagagtgttcgaaggactcggcgtggtaagctgagctaggagagggttgttcgaccactggctgttcgagtgactcgctgtagtaggcagaggacacagcttcctccaggttgtcagtggtcttgagcagacactccaccaaatcgttgtcagtgagcgagttaactgaggcgaggaagttgctagcggcagcggtttcagagtcggagatgacagtatcagctccgtccggggttgggtggttgtagtaagacaagtaatcgttaggttgcttgtcgcagaactccgagtatgagttgtcgaagctagcacgagagggagtgctggcagaggtgtaggaagcgttgaagttgatttgagtcatggtgacctggttgttcacgatcttatcgccacctgtgtccacctgcagttgctgggcctcagcgcaggctgaagtggcctcacaggagtaggggctggaagcacagttggaagtcatgatgttttcttggacgttcaggacgtggctggatgtacggatcatgcgcccgatggtgggacggtatgaataatccggaatatttataggtttttttattacaaaactgttacgaaaacagtaaaatacttatttatttgcgagatggttatcattttaattatctccatgatcggatctcctaggctcaagcagtgatcagatccagacatgataagatacattgatgagtttggacaaaccacaactagaatgcagtgaaaaaaatgctttatttgtgaaatttgtgatgctattgctttatttgtaaccattataagctgcaataaacaagttaacaacaacaattgcatttgtctagtacttctcgacggtaccgcatgctatgcatcagctgctagcaccatggctcgagttacagattacgagtcaggtatctggtgccaatggggcgaggctctgaatacacgccattagtgtccacagtaaagtccacattaacagacttgttgtagttggaagtgtactgaatttcgggattccagcgtttgctgttttccttctgcagctcccactcgatctccacgctgacctgtcccgtggagtactgtgtgatgaaggaagcaaactttgccgcactgaaggtggtcgaaggattcgcaggtaccggggtgttcttgatgagaatctgtggaggagggtgtttaagtccgaatccacccatgaggggagaggggtgaaaatgtccgtccgtgtgtggaatctttgcccagatgggcccctgaaggtacacatctctgtcctgccagaccatgcctggaagaacgccttgtgtgttgacatctgcggtagctgcttgtctgttgcctctctggaggttggtagatacagaaccatactgctccgtagccacgggattggttgtcctgatttcctcttcgtctgtaatcatgaccttttcaatgtccacatttgttttctctgagccttgcttcccaaagatgagaaccccgctctgaggaaaaaacttttcttcatcgtccttgtggcttgccatcgccgggcccggattcaccagagagtctctgccattgaggtggtacttggtagctccagtccacgagtattcactgttgttgttatccgcagatgtctttgatactcgctgctggcggtaacagggtccaggaagccagttcctagactggtcccgaatgtcactcgctccggcctgagaaaactgaagccttgactgcgtggtggttccacttggagtgtttgttctgctcaagtaatacaggtactggtcgatgagaggattcatgagacggtccagactctggctgtgagcgtagctgctgtggaaaggaacgtcctcaaaagtgtagctgaaggtaaagttgtttccggtacgcagcatctgagaaggaaagtactccaggcagtaaaatgaagagcgtcctactgcctgactcccgttgttcagggtgaggtatccatactgtggcaccatgaagacgtctgctgggaacggcgggaggcatccttgatgcgccgagccgaggacgtacgggagctggtactccgagtcagtaaacacctgaaccgtgctggtaaggttattggcaatcgtcgtcgtaccgtcattctgcgtgacctctttgacttgaatgttaaagagcttgaagttgagtctcttgggtcggaatccccagttgttgttgatgagtctttgccagtcacgtggtgaaaagtggcagtggaatctgttgaagtcaaaatacccccaaggggtgctgtagccaaagtagtgattgtcgttcgaggctcctgattggctggaaatttgtttgtagaggtggttgttgtaggtgggcagggcccaggttcgggtgctggtggtgatgactctgtcgcccatccatgtggaatcgcaatgccaatttcccgaggaattacccactccgtcggcgccctcgttattgtctgccattggtgcgccactgcctgtagccatcgtattagttcccagaccagagggggctgctggtggctgtccgagaggctgggggtcaggtactgagtctgcgtctccagtctgaccaaaattcaatctttttcttgcaggctgctggcccgcctttccggttcccgaggaggagtctggctccacaggagagtgctctaccggcctcttttttcccggagccgtcttaacaggttcctcaaccaggcccagaggttcaagaaccctctttttcgcctggaagactgctcgtccgaggttgcccccaaaagacgtatcttctttaaggcgctcctggaactccgcgtcggcgtggttgtacttgaggtaagggttgtctccgctgtcgagctgccggtcgtaggctttgtcgtgctcgagggcagcggcgtctgcctcgttcaccggctctcccttgtccagtccgttgaagggtccgaggtacttgtacccgggaagcacaaggcccctgctgtcgtccttatgccgctctgcgggctttggtggtggtgggccgggtttgagcttccaccactgtcttattccttcagagagagtgtcctcgagccaatcgggtagataaccgtcggcagccgtggcggctcaagtcttcgtcgagtgattgtaaataaaatgtaatttacagtatagtattttaattaatatacaaatgatttgataataattcttatttaactataatatattgtgttgggttgaattaaaggtccgtatctccagactgcagtttaaattgtgtaatttatgtagctgtaatttttaccttattaatattttttacgctttgcattcgacgactgaactcccaaatatatgtttaactcgtcttggtcgtttgaatttttgttgctgtgtttcctaatattttccatcaccttaaatatgttattgtaatcctcaatgttgaacttgcaattggacacggcatagttttccatagtcgtgtaaaacatggtattggctgcattgtaatacatccgactgagcgggtacggatctatgtgtttgagcagcctgttcaaaaactctgcatcgtcgcaaaacggaatttggtcacgatcccggtccgaagcgcgcggaattcaaagcgctacgtcagcgacgtcatcgattattgctccaatactagggttttgttttactatctgttctgcggtccacacatcttcttcgctagtcacgtacgcaaacaactcgggccgcaaaggtgttttaaaacatatcagattagaatcttttataacttggccgcattgtaaatagttgtgccaacgcgcgggaaacattttacacgtgctttcaatcttatctcataaacgcaactaaatatgatccttcaactcgctttacgagtagaattctacttgtaacgcacgattaattatgactcataagctgatgtcatgttttgcacacggctcataaccgaactcgctttacgagtagaattctacgcgtaaaacacaatcaagtatgagtcataagctgatgtcatgttttgcacacggctcataaccgaactggctttacgagtagaattctacttgtaacgcacgatcagtggatgatgtcataaacttatctcatgttttgcacacggctcataacttgagtcataagctgatatcagaagattattaacgtgtttaggtatgactcatttgttttcaaaactgaactcgctttacggatagaattctacttgtaaaacacaatcaggggatgatgtcattatacaaatgatgtcatttgtttttcaaaactaaactcgctttacgggtagaattctacttgtaaaacacaatcgagggataatgtcatttgttattctcaaatatgatgtcatttaaatttttattatgcaagaattgtatgttgctgtgtcatttatgaatgttttatcgacaacttgtttatttgtttcattgacttgttgttgttcgtgattatgattaattataaatcttttgttggggtcaacatcgatgtatacgccgctacagggcgcgtactatggttgctttgacgtatgcggtgtgaaataccgcacagatgcgtaaggagaaaataccgcatcaggcgcccctgcaggcagctgcgcgctcgctcgctcactgaggccgcccgggcaaagcccgggcgtcgggcgacctttggtcgcccggcctcagtgagcgagcgagcgcgcagagagggagtggccaactccatcactaggggttcctacgcgttagttattaatagtaatcaattacggggtcattagttcatagcccatatatggagttccgcgttacataacttacggtaaatggcccgcctggctgaccgcccaacgacccccgcccattgacgtcaataatgacgtatgttcccatagtaacgccaatagggactttccattgacgtcaatgggtggagtatttacggtaaactgcccacttggcagtacatcaagtgtatcatatgccaagtacgccccctattgacgtcaatgacggtaaatggcccgcctggcattatgcccagtacatgaccttatgggactttcctacttggcagtacatctacgtattagtcatcgctattaccatggtgatgcggttttggcagtacatcaatgggcgtggatagcggtttgactcacggggatttccaagtctccaccccattgacgtcaatgggagtttgttttggcaccaaaatcaacgggactttccaaaatgtcgtaacaactccgccccattgacgcaaatgggcggtaggcgtgtacggtgggaggtctatataagcagagctggtttagtgaaccgtcagatccgctagcgctaccggtcgccaccatggtgagcaagggcgaggagctgttcaccggggtggtgcccatcctggtcgagctggacggcgacgtaaacggccacaagttcagcgtgtccggcgagggcgagggcgatgccacctacggcaagctgaccctgaagttcatctgcaccaccggcaagctgcccgtgccctggcccaccctcgtgaccaccctgacctacggcgtgcagtgcttcagccgctaccccgaccacatgaagcagcacgacttcttcaagtccgccatgcccgaaggctacgtccaggagcgcaccatcttcttcaaggacgacggcaactacaagacccgcgccgaggtgaagttcgagggcgacaccctggtgaaccgcatcgagctgaagggcatcgacttcaaggaggacggcaacatcctggggcacaagctggagtacaactacaacagccacaacgtctatatcatggccgacaagcagaagaacggcatcaaggtgaacttcaagatccgccacaacatcgaggacggcagcgtgcagctcgccgaccactaccagcagaacacccccatcggcgacggccccgtgctgctgcccgacaaccactacctgagcacccagtccgccctgagcaaagaccccaacgagaagcgcgatcacatggtcctgctggagttcgtgaccgccgccgggatcactctcggcatggacgagctgtacaagtaggtcgacgtttatttgtgaaatttgtgatgctattgctttatttgtaaccatctagctttatttgtgaaatttgtgatgctattgctttatttgtaaccattataagctgcaataaacaagttaacaacaacaattgcattcattttatgtttcaggttcagggggagatgtgggaggttttttaaagtttaaacaggaacccctagtgatggagttggccactccctctctgcgcgctcgctcgctcactgaggccgggcgaccaaaggtcgcccgacgcccgggcggcctcagtgagcgagcgagcgcgcagctgcctgcaggacatgtgagcaaaaggccagcaaaaggccaggaaccgtaaaaaggccgcgttgctggcgtttttccataggctccgcccccctgacgagcatcacaaaaatcgacgctcgcggccgctctagagatcatggagataattaaaatgataaccatctcgcaaataaataagtattttactgttttcgtaacagttttgtaataaaaaaacctataaatattccggattattcataccgtcccaccatcgggcgcggatccgccgccctggcggggttttacgagattgtgattaaggtccccagcgaccttgacgagcatctgcccggcatttctgacagctttgtgaactgggtggccgagaaggagtgggagttgccgccagattctgacttggatctgaatctgattgagcaggcacccctgaccgtggccgagaagctgcagcgcgactttctgacggagtggcgccgtgtgagtaaggccccggaggcccttttctttgtgcaatttgagaagggagagagctacttccacttacacgtgctcgtggaaaccaccggggtgaaatccttagttttgggacgtttcctgagtcagattcgcgaaaaactgattcagagaatttaccgcgggatcgagccgactttgccaaactggttcgcggtcacaaagaccagaaacggcgccggaggcgggaacaaggtggtggacgagtgctacatccccaattacttgctccccaaaacccagcctgagctccagtgggcgtggactaatttagaacagtatttaagcgcctgtttgaatctcacggagcgtaaacggttggtggcgcagcatctgacgcacgtgtcgcagacgcaggagcagaacaaagagaatcagaatcccaattctgacgcgccggtgatcagatcaaaaacttcagccaggtacatggagctggtcgggtggctcgtggacaaggggattacctcggagaagcagtggatacaggaggaccaggcctcatacatctccttcaatgcggcctccaactcgcggtcccaaatcaaggctgccttggacaatgcgggaaagattatgagcctgactaaaaccgcccccgactacctggtgggccagcagcccgtggaggacatttccagcaatcggatttataaaattttggaactaaacgggtacgatccccaatatgcggcttccgtctttctgggatgggccacgaaaaagttcggcaagaggaacaccatctggctgtttgggcctgcaactaccgggaagaccaacatcgcggaggccatagcccacactgtgcccttctacgggtgcgtaaactggaccaatgagaactttcccttcaacgactgtgtggacaagatggtgatctggtgggaggaggggaagatgaccgccaaggtcgtggagtcggccaaagccattctcggaggaagcaaggtgcgcgtggaccagaaatgcaagtcctcggcccagatagacccgactcccgtgatcgtcacctccaacaccaacatgtgcgccgtgattgacgggaactcaacgaccttcgaacaccagcagccgttgcaagaccggatgttcaaatttgaactcacccgccgtctggatcatgactttgggaaggtcaccaagcaggaagtcaaagactttttccggtgggcaaaggatcacgtggttgaggtggagcatgaattctacgtcaaaaagggtggagccaagaaaagacccgcccccagtgacgcagatataagtgagcccaaacgggtgcgcgagtcagttgcgcagccatcgacgtcagacgcggaagcatcgatcaactacgcagacaggtaccaaaacaaatgttctcgtcacgtgggcatgaatctgatgctgtttccctgcagacaatgcgagagaatgaatcagaattcaaatatctgcttcactcacggacagaaagactgtttagagtgctttcccgtgtcagaatctcaacccgtttctgtcgtcaaaaaggcgtatcagaaactgtgctacattcatcatatcatgggaaaggtgccagacgcttgcactgcctgcgatctggtcaatgtggatttggatgactgcatctttgaacaataatctagagcctgcagtctcgacaagcttgtcgagaagtactagaggatcataatcagccataccacatttgtagaggttttacttgctttaaaaaacctcccacacctccccctgaacctgaaacataaaatgaatgcaattgttgttgttaacttgtttattgcagcttataatggttacaaataaagcaatagcatcacaaatttcacaaataaagcatttttttcactgcattctagttgtggtttgtccaaactcatcaatgtatcttatcatgtctggatctgatcactgcttgagcctaggagatccgaaccagataagtgaaatctagttccaaactattttgtcatttttaattttcgtattagcttacgacgctacacccagttcccatctattttgtcactcttccctaaataatccttaaaaactccatttccacccctcccagttcccaactattttgtccgcccacagcggggcatttttcttcctgttatgtttttaatcaaacatcctgccaactccatgtgacaaaccgtcatcttcggctacttt

SEQ ID NO: 10 - DNA, 786 bp, Unknown
  Nucleotide sequence of Acie0
atgataagaaccagcagtcacgtgctgaacgtccaggaaaatataatgacgtcaaactgtgcgtcatcgccatattcgtgcgaggcaacgtccgcttgcgcagaagctcagcaggtaatgatcgataactttgttttctttcacatgtacaacgccgacatacaaattgacgcaaagctgcaatgcggcgtgcgctcggccgcgtttgcaatgatcgacgataaacatttggaaatgtacaagcatagaatagagaataaatttttttattactatgatcaatgtgccgacattgccaaacccgaccgtctgcccgatgacgacggcgcgtgctgtcaccattttatttttgatgcccaacgtattattcaatgtattaaagagattgaaagcgcgtacggcgtgcgtgatcgcggcaatgtaatagtgttttatccgtacttgaaacagttgcgagacgcgttgaagctaattaaaaactcttttgcgtgttgttttaaaattataaattctatgcaaatgtacgtgaacgagttaatatcaaattgcctgttgtttattgaaaagctggaaactattaataaaactgttaaagttatgaatttgtttgtagacaatttggttttgtacgaatgcaatgtttgtaaagaaatatctacggatgaaagatttttaaagccaaaagaatgttgcgaatacgctatatgcaacgcgtgctgcgttaacatgtggaagacggccaccacgcacgcaaaatgtccagcgtgcaggacatcgtataaataa

SEQ ID NO: 11 - protein, 261 aa, Unknown
  Amino acid sequence of IE0 protein
MIRTSSHVLNVQENIMTSNCASSPYSCEATSACAEAQQVMIDNFVFFHMYNADIQIDAKLQCGVRSAAFAMIDDKHLEMYKHRIENKFFYYYDQCADIAKPDRLPDDDGACCHHFIFDAQRIIQCIKEIESAYGVRDRGNVIVFYPYLKQLRDALKLIKNSFACCFKIINSMQMYVNELISNCLLFIEKLETINKTVKVMNLFVDNLVLYECNVCKEISTDERFLKPKECCEYAICNACCVNMWKTATTHAKCPACRTSYK

SEQ ID NO: 12 - DNA, 1911 bp, Unknown
  Nucleotide sequence of Acie01
atgatccgtacatccagccacgtcctgaacgtccaagaaaacatcatgacttccaactgtgcttccagcccctactcctgtgaggccacttcagcctgcgctgaggcccagcaactgcaggtggacacaggtggcgataagatcgtgaacaaccaggtcaccatgactcaaatcaacttcaacgcttcctacacctctgccagcactccctctcgtgctagcttcgacaactcatactcggagttctgcgacaagcaacctaacgattacttgtcttactacaaccacccaaccccggacggagctgatactgtcatctccgactctgaaaccgctgccgctagcaacttcctcgcctcagttaactcgctcactgacaacgatttggtggagtgtctgctcaagaccactgacaacctggaggaagctgtgtcctctgcctactacagcgagtcactcgaacagccagtggtcgaacaaccctctcctagctcagcttaccacgccgagtccttcgaacactctgctggtgtcaaccagccgtcggccacaggcaccaagaggaagttggacgagtacctggataactcccagggagttgtgggtcaattcaacaagatcaagttgagacctaagtacaagaagagcaccatccagtcatgcgctacactggaacaaaccatcaaccacaacactaacatctgtacagtggcttccacccaggagatcactcactacttcacaaacgacttcgccccctacctgatgaggttcgacgataacgactacaactcgaacagattctccgatcacatgtctgaaaccggttactacatgttcgtcgttaagaagtccgaggtgaagcctttcgaaatcatcttcgccaagtacgtctctaacgtggtctacgagtacacaaacaactactacatggttgacaaccgtgtgttcgttgtgaccttcgataagatccgcttcatgatcagctacaacctggttaaggagactggcatcgaaatcccacactcacaggacgtctgcaacgatgagaccgccgctcaaaactgcaagaagtgtcacttcgtggacgtccaccacacattcaaggccgctctgacctcctacttcaacctcgatatgtactacgctcagacaaccttcgtgaccttgctgcaatcactcggcgagcgtaagtgtggattcctcttgtcgaagttgtacgagatgtaccaggacaagaacctcttcactttgcccatcatgctgagccgcaaggaatcaaacgagatcgaaaccgcctctaacaacttcttcgtctcgccatacgtttcccagatcctcaagtactcggagtccgtccaattcccggacaaccctcccaacaagtacgtcgttgataacctgaacctcatcgtgaacaagaagagcactctgacatacaagtactcgtccgtcgctaacctgctcttcaacaactacaagtaccacgacaacatcgcttctaacaacaacgccgagaacctcaagaaggtcaagaaggaagacggaagcatgcacatcgttgagcagtacttgactcaaaacgtcgataacgttaagggtcacaacttcatcgtgttgtccttcaagaacgaggaaaggctgaccatcgctaagaagaacaaggagttctactggatctctggcgaaatcaaggacgttgatgtgagccaggtcatccaaaagtacaacagattcaagcaccacatgttcgtgatcggcaaggtcaaccgtcgcgagtcaactacactgcacaacaacttgctgaagctcttggccttgatcctgcagggactggtgccactctccgacgccatcacattcgccgagcaaaagctcaactgcaagtacaagaagttcgagttcaactaa

SEQ ID NO: 13 - protein, 636 aa, Unknown
  Amino acid sequence of IE1 protein
MIRTSSHVLNVQENIMTSNCASSPYSCEATSACAEAQQLQVDTGGDKIVNNQVTMTQINFNASYTSASTPSRASFDNSYSEFCDKQPNDYLSYYNHPTPDGADTVISDSETAAASNFLASVNSLTDNDLVECLLKTTDNLEEAVSSAYYSESLEQPVVEQPSPSSAYHAESFEHSAGVNQPSATGTKRKLDEYLDNSQGVVGQFNKIKLRPKYKKSTIQSCATLEQTINHNTNICTVASTQEITHYFTNDFAPYLMRFDDNDYNSNRFSDHMSETGYYMFVVKKSEVKPFEIIFAKYVSNVVYEYTNNYYMVDNRVFVVTFDKIRFMISYNLVKETGIEIPHSQDVCNDETAAQNCKKCHFVDVHHTFKAALTSYFNLDMYYAQTTFVTLLQSLGERKCGFLLSKLYEMYQDKNLFTLPIMLSRKESNEIETASNNFFVSPYVSQILKYSESVQFPDNPPNKYVVDNLNLIVNKKSTLTYKYSSVANLLFNNYKYHDNIASNNNAENLKKVKKEDGSMHIVEQYLTQNVDNVKGHNFIVLSFKNEERLTIAKKNKEFYWISGEIKDVDVSQVIQKYNRFKHHMFVIGKVNRRESTTLHNNLLKLLALILQGLVPLSDAITFAEQKLNCKYKKFEFN

SEQ ID NO: 14 - DNA, 1227 bp, Unknown
  Nucleotide sequence of Acie02
atgagtcgccaaatcaacgccgccactcccagcagcagccgccgccacaggctgtctctcagccgtcgccgcatcaactttacaacatctcccgaagcccagccgtcttcaagcagtcgcagccagccgtcttcaagcagtcgcagccatcgccgtcaggagcggcgtcaggagcagcgtgtcagcgaagaaaacgtgcagattatcgggaacgtcaacgagccgttgacgcgcacctaccatcgtcagggtgtcacgtattacgtgcacggtcaggttaacattagcaatgacgatccgctattaagtcaagaggatgacgtcatactaattaatagtgaaaatgtggatcgtgaacggtttcccgacatcactgcccagcagtaccaggataacattgcgtcggagacagctgcgcagagggctctgcaacgaggtttagatcttgaggctcagctgatgaatgagattgccccaaggtctcccacttatagtccatcttattcgccgaattacgtaataccacagtcgccagatttgtttgcctcgccgcagtctccgcagccgcagcagcagcagcagcagcaatcagaacccgaagaagaagtagaggtttcgtgtaatatttgttttactacttttaaagacactaaaaacgtaaattcctcgtttgtgacttcgattcattgtaaccatgctgtgtgtttcaagtgttatgtcaagataattatggacaattctgtgtacaaatgtttttgcagcgctacttcatcagattgtcgcgtgtacaataagcacgggtatgtagaatttatgcccattaacgtcactcgtaaccaggattccatcaaacagcattggcgcgagcttttagaaaataacacggtcaacaatcacaccacggacttgaactatgtggagcaattgcaaaaagaactgtccgagctgcgagccaagaccagccaagttgaacataaaatgaccatgttaaacagcgactacattatgcttaaacacaagcatgctgtcgccgaattagatttacaaaaggcaaactatgacttgcaagaatctaccaagaaatcagaagagttgcaatcgactgtgaataatctgcaagaacaattgcgtaagcaggtggccgagtctcaagccaaattttcagagtttgagcgcagtaactctgatttagtttctaagttacaaactgttatgtctagacgttaa

SEQ ID NO: 15 - protein, 408 aa, Unknown
  Amino acid sequence of IE2 protein
MSRQINAATPSSSRRHRLSLSRRRINFTTSPEAQPSSSSRSQPSSSSRSHRRQERRQEQRVSEENVQIIGNVNEPLTRTYHRQGVTYYVHGQVNISNDDPLLSQEDDVILINSENVDRERFPDITAQQYQDNIASETAAQRALQRGLDLEAQLMNEIAPRSPTYSPSYSPNYVIPQSPDLFASPQSPQPQQQQQQQSEPEEEVEVSCNICFTTFKDTKNVNSSFVTSIHCNHAVCFKCYVKIIMDNSVYKCFCSATSSDCRVYNKHGYVEFMPINVTRNQDSIKQHWRELLENNTVNNHTTDLNYVEQLQKELSELRAKTSQVEHKMTMLNSDYIMLKHKHAVAELDLQKANYDLQESTKKSEELQSTVNNLQEQLRKQVAESQAKFSEFERSNSDLVSKLQTVMSRR

SEQ ID NO: 16 - DNA, 881 bp, Unknown
  Nucleotide sequence of hr1 of baculovirus
atcgatgttgaccccaacaaaagatttataattaatcataatcacgaacaacaacaagtcaatgaaacaaataaacaagttgtcgataaaacattcataaatgacacagcaacatacaattcttgcataataaaaatttaaatgacatcatatttgagaataacaaatgacattatccctcgattgtgttttacaagtagaattctacccgtaaagcgagtttagttttgaaaaacaaatgacatcatttgtataatgacatcatcccctgattgtgttttacaagtagaattctatccgtaaagcgagttcagttttgaaaacaaatgagtcatacctaaacacgttaataatcttctgatatcagcttatgactcaagttatgagccgtgtgcaaaacatgagataagtttatgacatcatccactgatcgtgcgttacaagtagaattctactcgtaaagccagttcggttatgagccgtgtgcaaaacatgacatcagcttatgactcatacttgattgtgttttacgcgtagaattctactcgtaaagcgagttcggttatgagccgtgtgcaaaacatgacatcagcttatgagtcataattaatcgtgcgttacaagtagaattctactcgtaaagcgagttgaaggatcatatttagttgcgtttatgagataagattgaaagcacgtgtaaaatgtttcccgcgcgttggcacaactatttacaatgcggccaagttataaaagattctaatctgatatgttttaaaacacctttgcggcccgagttgtttgcgtacgtgactagcgaagaagatgtgtggaccgcagaacagatagtaaaacaaaaccctagtattggagcaataatcgat

SEQ ID NO: 17 - DNA, 990 bp, Unknown
  Nucleotide sequence of hr2 of baculovirus
tgagcaaaacacaaccggcaaattctcggcggccgtttgggaatgcggaataattgccatatgtaaatgatgtcatcggttctaactcgctttacgagtagaattctacgtgtaaaacataatcaagagatgatgtcatttgtttttcaaaactgaactcaagaaatgatgtcatttgtttttcaaaactgaactggctttacgagtagaattctacttgtaaaacacaatcgagagatgatgtcatattttgcacacggctctaattaaactcgctttacgagtaaaattctacttgtaacgcatgatcaagggatgatgtcattggatgagtcatttgtttttcaaaactaaactcgctttacgagtagaattctacttgtaaaacacaatcaagggatgatgtcattatacaaatgatgtcatttgtttttcaaaactaaactcgctttacgggtagaattctacttgtaaaacagcaactcgagggatgatgtcatcctttactcgatgattataaacgtgtttatgtatgactcatttgtttttcaaaactaaactcgctttacgagtagaattctacttgtaacgcacgatcaagggatgatgtcatttatttgtgcaaagctcgatgtcatcttttgcacacgattataaacacaatccaaataatgactcatttgttttcaaaactgaactcgctttacgagtagaattctacttgtaaaacacaatcaagggatgatgtcattttcaaaatgatgtcatttgtttttcaaaactaaactcgctttacgagtagaattctacttgtaaaacacaatcaagggatgatgtcattttaaaaatgatcatttgtttttcaaaactaaactcgctttacgagtagaattctacgtgtaaaacacaatcaagggatgatgtcatttactaaataaaataattatttaaataaaactgttttttattgtcaaatacacattgattcac

SEQ ID NO: 18 - DNA, 684 bp, Unknown
  Nucleotide sequence of hr3 of baculovirus
acgcgtagaattctacttgtaaagcaagttaaaataagccgtgtgcaaaaatgacatcagacaaatgacatcatctacctatcatgatcatgttaataatcatgttttaaaatgacatcagcttatgactaataattgatcgtgcgttacaagtagaattctactcgtaaagcgagtttagttttgaaaacaaatgagtcatcattaaacatgttaataatcgtgtataaaggatgacatcatccactaatcgtgcgttacaagtagaattctactcgtaaagcgagttcggttttgaaaaacaaatgacatcatttcttgattgtgttttacacgtagaattctactcgtaaagtatgttcagtttaaaaaacaaatgacatcattttacagatgacatcatttcttgattatgttttacaagtagaattctactcgtaaagcgagtttagttttaaaaaacaaatgacatcatctcttgattatgttttacaagtagaattctactcgtaaagcgagtttagttttgaaaaacaaatgacatcatctcttgattatgttttacaagtagaattctactcgtaaagcgagtttagttttgaaaaacaaatgacatcatcccttgatcatgcgttacaagtagaattctactcgtaaagcgagttgaattttgattacaatatt

SEQ ID NO: 19 - DNA, 675 bp, Unknown
  Nucleotide sequence of hr4 left of baculovirus
atgcatataattgtgtacaaaatatgactcattaatcgatcgtgcgttacaagtagaattctactggtaaagcaagttcggttgtgagccgtgtgcaaaacatgacatcataactaatcatgtttataatcatgtgcaaaatatgacatcatccgacgattgtgttttacaagtagaattctactcgtaaagcgagtttaaaaattttgtgacgtcaatgaaacaacgtgtaatattttttacaatatttaagtgaaacattatgacttccaataattttgtggatgtggatacgtttgcaagacaattgattacagataaatgtagtgctctaatcgaaagatgcggatctgttgccggcaaacattttagagattagtagagaaaggccagagacaagtattttgaggtgccaactcaaaaaaactatgaatacattaaaaaattatttttacgaacaaaatatatggacgattcgatagattataaagattttaacagacgcatcctattgatagtttttaaattcgctttaaacaagagcaccaactactttccatcgtactaaagagatcatcgaggtggccattaaacgtttaaacaaaattaaccccgatttaaagagttctccgcgcaatgcttcagcattacaaatgaatgtttggaaaatctaga

SEQ ID NO: 20 - DNA, 418 bp, Unknown
  Nucleotide sequence of hr4 right of baculovirus
aactggctttacgagtagaattctacttgtaaaacacaatcaagaaatgatgtcatttttgtacgtgattataaacatgtttaaacatggtacattgaacttaatttttgcaagttgataaactagattaatgtatgactcatttgtttgtgcaagttgataaacgtgattaatatatgactcatatgtttgtgcaaaaatggtgtcatcgtacaaactcgctttacgagtagaattctacttgtaaaacacaatcgagggatgatgtcatttgtagaatgatgtcatttgttttttcaaaaccgaactcgctttacgagtagaattctacttgtaaaacacaatcgagggatgatgtcatttgtagaatgatgtcatcgtacaaactcgctttacgagtagaattctagtaaaacac

SEQ ID NO: 21 - DNA, 725 bp, Unknown
  Nucleotide sequence of hr5 of baculovirus
ttgaaaatttattgcctaatattatttttgtcagttcgttgtcatttattaatttggatgatgtccatttgtttttaaaattgaactggctttacgagtagaattctacgcgtaaaacacaatcaagtatgagtcataagctgatgtcatgttttgcacacggctcataaccgaactggctttacgagtagaattctacttgtaacgcacgatcgagtggatgatggtcatttgtttttcaaatcgagatgatgtcatgttttgcacacgggctcataaactgctttacgagtagaattctacgtgtaacgcacgatcgattgatgagtcatttgttttgcaatatgatatcatacaatatgactcatttgtttttcaaaaccgaacttgatttacgggtagaattctactcgtaaagcacaatcaaaaagatgatgtcatttgtttttcaaaactgaactctcggctttacgagtagaattctacgtgtaaaacacaatcaagaaatgatgtcatttgttataaaaataaaagctgatgtcatgttttgcacatggctcataactaaactcgctttacgggtagaattctacgcgtaaaacatgattgataattaaataattcatttgcaaagctatacgttaaatcaaacggacgttatggaattgtataatattaaatatgcaattgatccaacaaataaaattataatagagcaagtcgac

SEQ ID NO: 22 - DNA, 4400 bp, Artificial sequence
  pAAV-EGFP plasmid
acatgtgagcaaaaggccagcaaaaggccaggaaccgtaaaaaggccgcgttgctggcgtttttccataggctccgcccccctgacgagcatcacaaaaatcgacgctcaagtcagaggtggcgaaacccgacaggactataaagataccaggcgtttccccctggaagctccctcgtgcgctctcctgttccgaccctgccgcttaccggatacctgtccgcctttctcccttcgggaagcgtggcgctttctcatagctcacgctgtaggtatctcagttcggtgtaggtcgttcgctccaagctgggctgtgtgcacgaaccccccgttcagcccgaccgctgcgccttatccggtaactatcgtcttgagtccaacccggtaagacacgacttatcgccactggcagcagccactggtaacaggattagcagagcgaggtatgtaggcggtgctacagagttcttgaagtggtggcctaactacggctacactagaaggacagtatttggtatctgcgctctgctgaagccagttaccttcggaaaaagagttggtagctcttgatccggcaaacaaaccaccgctggtagcggtggtttttttgtttgcaagcagcagattacgcgcagaaaaaaaggatctcaagaagatcctttgatcttttctacggggtctgacgctcagtggaacgaaaactcacgttaagggattttggtcatgagattatcaaaaaggatcttcacctagatccttttaaattaaaaatgaagttttaaatcaatctaaagtatatatgagtaaacttggtctgacagttaccaatgcttaatcagtgaggcacctatctcagcgatctgtctatttcgttcatccatagttgcctgactccccgtcgtgtagataactacgatacgggagggcttaccatctggccccagtgctgcaatgataccgcgagacccacgctcaccggctccagatttatcagcaataaaccagccagccggaagggccgagcgcagaagtggtcctgcaactttatccgcctccatccagtctattaattgttgccgggaagctagagtaagtagttcgccagttaatagtttgcgcaacgttgttgccattgctacaggcatcgtggtgtcacgctcgtcgtttggtatggcttcattcagctccggttcccaacgatcaaggcgagttacatgatcccccatgttgtgcaaaaaagcggttagctccttcggtcctccgatcgttgtcagaagtaagttggccgcagtgttatcactcatggttatggcagcactgcataattctcttactgtcatgccatccgtaagatgcttttctgtgactggtgagtactcaaccaagtcattctgagaatagtgtatgcggcgaccgagttgctcttgcccggcgtcaatacgggataataccgcgccacatagcagaactttaaaagtgctcatcattggaaaacgttcttcggggcgaaaactctcaaggatcttaccgctgttgagatccagttcgatgtaacccactcgtgcacccaactgatcttcagcatcttttactttcaccagcgtttctgggtgagcaaaaacaggaaggcaaaatgccgcaaaaaagggaataagggcgacacggaaatgttgaatactcatactcttcctttttcaatattattgaagcatttatcagggttattgtctcatgagcggatacatatttgaatgtatttagaaaaataaacaaataggggttccgcgcacatttccccgaaaagtgccacctgacgtctaagaaaccattattatcatgacattaacctataaaaataggcgtatcacgaggccctttcgtctcgcgcgtttcggtgatgacggtgaaaacctctgacacatgcagctcccggagacggtcacagcttgtctgtaagcggatgccgggagcagacaagcccgtcagggcgcgtcagcgggtgttggcgggtgtcggggctggcttaactatgcggcatcagagcagattgtactgagagtgcaccataaaattgtaaacgttaatattttgttaaaattcgcgttaaatttttgttaaatcagctcattttttaaccaataggccgaaatcggcaaaatcccttataaatcaaaagaatagcccgagatagggttgagtgttgttccagtttggaacaagagtccactattaaagaacgtggactccaacgtcaaagggcgaaaaaccgtctatcagggcgatggcccactacgtgaaccatcacccaaatcaagttttttggggtcgaggtgccgtaaagcactaaatcggaaccctaaagggagcccccgatttagagcttgacggggaaagccggcgaacgtggcgagaaaggaagggaagaaagcgaaaggagcgggcgctagggcgctggcaagtgtagcggtcacgctgcgcgtaaccaccacacccgccgcgcttaatgcgccgctacagggcgcgtactatggttgctttgacgtatgcggtgtgaaataccgcacagatgcgtaaggagaaaataccgcatcaggcgcccctgcaggcagctgcgcgctcgctcgctcactgaggccgcccgggcaaagcccgggcgtcgggcgacctttggtcgcccggcctcagtgagcgagcgagcgcgcagagagggagtggccaactccatcactaggggttcctacgcgttagttattaatagtaatcaattacggggtcattagttcatagcccatatatggagttccgcgttacataacttacggtaaatggcccgcctggctgaccgcccaacgacccccgcccattgacgtcaataatgacgtatgttcccatagtaacgccaatagggactttccattgacgtcaatgggtggagtatttacggtaaactgcccacttggcagtacatcaagtgtatcatatgccaagtacgccccctattgacgtcaatgacggtaaatggcccgcctggcattatgcccagtacatgaccttatgggactttcctacttggcagtacatctacgtattagtcatcgctattaccatggtgatgcggttttggcagtacatcaatgggcgtggatagcggtttgactcacggggatttccaagtctccaccccattgacgtcaatgggagtttgttttggcaccaaaatcaacgggactttccaaaatgtcgtaacaactccgccccattgacgcaaatgggcggtaggcgtgtacggtgggaggtctatataagcagagctggtttagtgaaccgtcagatccgctagcgctaccggtcgccaccatggtgagcaagggcgaggagctgttcaccggggtggtgcccatcctggtcgagctggacggcgacgtaaacggccacaagttcagcgtgtccggcgagggcgagggcgatgccacctacggcaagctgaccctgaagttcatctgcaccaccggcaagctgcccgtgccctggcccaccctcgtgaccaccctgacctacggcgtgcagtgcttcagccgctaccccgaccacatgaagcagcacgacttcttcaagtccgccatgcccgaaggctacgtccaggagcgcaccatcttcttcaaggacgacggcaactacaagacccgcgccgaggtgaagttcgagggcgacaccctggtgaaccgcatcgagctgaagggcatcgacttcaaggaggacggcaacatcctggggcacaagctggagtacaactacaacagccacaacgtctatatcatggccgacaagcagaagaacggcatcaaggtgaacttcaagatccgccacaacatcgaggacggcagcgtgcagctcgccgaccactaccagcagaacacccccatcggcgacggccccgtgctgctgcccgacaaccactacctgagcacccagtccgccctgagcaaagaccccaacgagaagcgcgatcacatggtcctgctggagttcgtgaccgccgccgggatcactctcggcatggacgagctgtacaagtaggtcgacgtttatttgtgaaatttgtgatgctattgctttatttgtaaccatctagctttatttgtgaaatttgtgatgctattgctttatttgtaaccattataagctgcaataaacaagttaacaacaacaattgcattcattttatgtttcaggttcagggggagatgtgggaggttttttaaagtttaaacaggaacccctagtgatggagttggccactccctctctgcgcgctcgctcgctcactgaggccgggcgaccaaaggtcgcccgacgcccgggcggcctcagtgagcgagcgagcgcgcagctgcctgcagg